European Patent Application EP 4 495 234 A1, published January 22, 2025. Title: Variant of aspartate 1-decarboxylase derived from T. castaneum and microorganisms including the same. Applicant: CJ CheilJedang Corporation. The sequence listing filed with the application follows.

SEQUENCE LISTING (84 sequences)

SEQ ID NO: 1 - DNA, 35 bp, synthetic construct
  misc_feature 1..35: note = synthetic_primer
  source 1..35: mol_type = other DNA
agatcgaaaggtgcacaaagatgccggcaaccgga

SEQ ID NO: 2 - DNA, 26 bp, synthetic construct
  misc_feature 1..26: note = synthetic_primer
  source 1..26: mol_type = other DNA
ggtcgacagcgctccagagttgattt

SEQ ID NO: 3 - DNA, 28 bp, synthetic construct
  misc_feature 1..28: note = synthetic_primer
  source 1..28: mol_type = other DNA
tttgtaaatcaactctggagcgctgtcg

SEQ ID NO: 4 - DNA, 38 bp, synthetic construct
  misc_feature 1..38: note = synthetic_primer
  source 1..38: mol_type = other DNA
cgctctagaactagtggatcttacaaatctgaaccaag

SEQ ID NO: 5 - DNA, 26 bp, synthetic construct
  misc_feature 1..26: note = synthetic_primer
  source 1..26: mol_type = other DNA
ggtcgacagcgctatggagttgattt

SEQ ID NO: 6 - DNA, 28 bp, synthetic construct
  misc_feature 1..28: note = synthetic_primer
  source 1..28: mol_type = other DNA
tttgtaaatcaactccatagcgctgtcg

SEQ ID NO: 7 - DNA, 26 bp, synthetic construct
  misc_feature 1..26: note = synthetic_primer
  source 1..26: mol_type = other DNA
ggtcgacagcgctggtgagttgattt

SEQ ID NO: 8 - DNA, 28 bp, synthetic construct
  misc_feature 1..28: note = synthetic_primer
  source 1..28: mol_type = other DNA
tttgtaaatcaactcaccagcgctgtcg

SEQ ID NO: 9 - DNA, 26 bp, synthetic construct
  misc_feature 1..26: note = synthetic_primer
  source 1..26: mol_type = other DNA
ggtcgacagcgctagcgagttgattt

SEQ ID NO: 10 - DNA, 28 bp, synthetic construct
  misc_feature 1..28: note = synthetic_primer
  source 1..28: mol_type = other DNA
tttgtaaatcaactcgctagcgctgtcg

SEQ ID NO: 11 - DNA, 26 bp, synthetic construct
  misc_feature 1..26: note = synthetic_primer
  source 1..26: mol_type = other DNA
ggtcgacagcgctacagagttgattt

SEQ ID NO: 12 - DNA, 28 bp, synthetic construct
  misc_feature 1..28: note = synthetic_primer
  source 1..28: mol_type = other DNA
tttgtaaatcaactctgtagcgctgtcg

SEQ ID NO: 13 - DNA, 26 bp, synthetic construct
  misc_feature 1..26: note = synthetic_primer
  source 1..26: mol_type = other DNA
ggtcgacagcgctagggagttgattt

SEQ ID NO: 14 - DNA, 28 bp, synthetic construct
  misc_feature 1..28: note = synthetic_primer
  source 1..28: mol_type = other DNA
tttgtaaatcaactccctagcgctgtcg

SEQ ID NO: 15 - DNA, 26 bp, synthetic construct
  misc_feature 1..26: note = synthetic_primer
  source 1..26: mol_type = other DNA
ggtcgacagcgctagagagttgattt

SEQ ID NO: 16 - DNA, 28 bp, synthetic construct
  misc_feature 1..28: note = synthetic_primer
  source 1..28: mol_type = other DNA
tttgtaaatcaactctctagcgctgtcg

SEQ ID NO: 17 - DNA, 26 bp, synthetic construct
  misc_feature 1..26: note = synthetic_primer
  source 1..26: mol_type = other DNA
ggtcgacagcgctaaggagttgattt

SEQ ID NO: 18 - DNA, 28 bp, synthetic construct
  misc_feature 1..28: note = synthetic_primer
  source 1..28: mol_type = other DNA
tttgtaaatcaactccttagcgctgtcg

SEQ ID NO: 19 - DNA, 26 bp, synthetic construct
  misc_feature 1..26: note = synthetic_primer
  source 1..26: mol_type = other DNA
ggtcgacagcgctgatgagttgattt

SEQ ID NO: 20 - DNA, 28 bp, synthetic construct
  misc_feature 1..28: note = synthetic_primer
  source 1..28: mol_type = other DNA
tttgtaaatcaactcatcagcgctgtcg

SEQ ID NO: 21 - DNA, 26 bp, synthetic construct
  misc_feature 1..26: note = synthetic_primer
  source 1..26: mol_type = other DNA
ggtcgacagcgctccggagttgattt

SEQ ID NO: 22 - DNA, 28 bp, synthetic construct
  misc_feature 1..28: note = synthetic_primer
  source 1..28: mol_type = other DNA
tttgtaaatcaactccggagcgctgtcg

SEQ ID NO: 23 - DNA, 26 bp, synthetic construct
  misc_feature 1..26: note = synthetic_primer
  source 1..26: mol_type = other DNA
ggtcgacagcgcttttgagttgattt

SEQ ID NO: 24 - DNA, 28 bp, synthetic construct
  misc_feature 1..28: note = synthetic_primer
  source 1..28: mol_type = other DNA
tttgtaaatcaactcaaaagcgctgtcg

SEQ ID NO: 25 - DNA, 26 bp, synthetic construct
  misc_feature 1..26: note = synthetic_primer
  source 1..26: mol_type = other DNA
ggtcgacagcgctcacgagttgattt

SEQ ID NO: 26 - DNA, 28 bp, synthetic construct
  misc_feature 1..28: note = synthetic_primer
  source 1..28: mol_type = other DNA
tttgtaaatcaactcgtgagcgctgtcg

SEQ ID NO: 27 - DNA, 26 bp, synthetic construct
  misc_feature 1..26: note = synthetic_primer
  source 1..26: mol_type = other DNA
ggtcgacagcgctcatgagttgattt

SEQ ID NO: 28 - DNA, 28 bp, synthetic construct
  misc_feature 1..28: note = synthetic_primer
  source 1..28: mol_type = other DNA
tttgtaaatcaactcatgagcgctgtcg

SEQ ID NO: 29 - DNA, 26 bp, synthetic construct
  misc_feature 1..26: note = synthetic_primer
  source 1..26: mol_type = other DNA
ggtcgacagcgctatcgagttgattt

SEQ ID NO: 30 - DNA, 28 bp, synthetic construct
  misc_feature 1..28: note = synthetic_primer
  source 1..28: mol_type = other DNA
tttgtaaatcaactcgatagcgctgtcg

SEQ ID NO: 31 - DNA, 26 bp, synthetic construct
  misc_feature 1..26: note = synthetic_primer
  source 1..26: mol_type = other DNA
ggtcgacagcgctttcgagttgattt

SEQ ID NO: 32 - DNA, 28 bp, synthetic construct
  misc_feature 1..28: note = synthetic_primer
  source 1..28: mol_type = other DNA
tttgtaaatcaactcgaaagcgctgtcg

SEQ ID NO: 33 - DNA, 26 bp, synthetic construct
  misc_feature 1..26: note = synthetic_primer
  source 1..26: mol_type = other DNA
ggtcgacagcgctaccgagttgattt

SEQ ID NO: 34 - DNA, 28 bp, synthetic construct
  misc_feature 1..28: note = synthetic_primer
  source 1..28: mol_type = other DNA
tttgtaaatcaactcggtagcgctgtcg

SEQ ID NO: 35 - DNA, 26 bp, synthetic construct
  misc_feature 1..26: note = synthetic_primer
  source 1..26: mol_type = other DNA
ggtcgacagcgctgttgagttgattt

SEQ ID NO: 36 - DNA, 28 bp, synthetic construct
  misc_feature 1..28: note = synthetic_primer
  source 1..28: mol_type = other DNA
tttgtaaatcaactcaacagcgctgtcg

SEQ ID NO: 37 - DNA, 26 bp, synthetic construct
  misc_feature 1..26: note = synthetic_primer
  source 1..26: mol_type = other DNA
ggtcgacagcgctttggagttgattt

SEQ ID NO: 38 - DNA, 28 bp, synthetic construct
  misc_feature 1..28: note = synthetic_primer
  source 1..28: mol_type = other DNA
tttgtaaatcaactccaaagcgctgtcg

SEQ ID NO: 39 - DNA, 41 bp, synthetic construct
  misc_feature 1..41: note = synthetic_primer
  source 1..41: mol_type = other DNA
cttgatatcgaattcctgcattcagggtagttgactaaaga

SEQ ID NO: 40 - DNA, 17 bp, synthetic construct
  misc_feature 1..17: note = synthetic_primer
  source 1..17: mol_type = other DNA
ctttgtgcacctttcga

SEQ ID NO: 41 - DNA, 40 bp, synthetic construct
  misc_feature 1..40: note = synthetic_primer
  source 1..40: mol_type = other DNA
tgaattcgagctcggtacccgaaatagcgcttgatgaatc

SEQ ID NO: 42 - DNA, 40 bp, synthetic construct
  misc_feature 1..40: note = synthetic_primer
  source 1..40: mol_type = other DNA
ggttgctacctgcacccggggggcatgagtatagatgtga

SEQ ID NO: 43 - DNA, 40 bp, synthetic construct
  misc_feature 1..40: note = synthetic_primer
  source 1..40: mol_type = other DNA
ctatactcatgccccccgggtgcaggtagcaaccacaaag

SEQ ID NO: 44 - DNA, 40 bp, synthetic construct
  misc_feature 1..40: note = synthetic_primer
  source 1..40: mol_type = other DNA
gtcgactctagaggatcccctatgtggcgttgggtgcagc

SEQ ID NO: 45 - DNA, 35 bp, synthetic construct
  misc_feature 1..35: note = synthetic_primer
  source 1..35: mol_type = other DNA
catctatactcatgccccccttcagggtagttgac

SEQ ID NO: 46 - DNA, 35 bp, synthetic construct
  misc_feature 1..35: note = synthetic_primer
  source 1..35: mol_type = other DNA
ggtggtcggtttcatctttgtgcacctttcgatct

SEQ ID NO: 47 - DNA, 37 bp, synthetic construct
  misc_feature 1..37: note = synthetic_primer
  source 1..37: mol_type = other DNA
tagatcgaaaggtgcacaaagatgaaaccgaccacca

SEQ ID NO: 48 - DNA, 41 bp, synthetic construct
  misc_feature 1..41: note = synthetic_primer
  source 1..41: mol_type = other DNA
ccgctctagaactagtggatcttaatggaaactgtgttctt

SEQ ID NO: 49 - DNA, 20 bp, synthetic construct
  misc_feature 1..20: note = synthetic_primer
  source 1..20: mol_type = other DNA
cccacccggtgtcattcgac

SEQ ID NO: 50 - DNA, 19 bp, synthetic construct
  misc_feature 1..19: note = synthetic_primer
  source 1..19: mol_type = other DNA
gcgcatccagctcatcggt

SEQ ID NO: 51 - protein, 540 aa, synthetic construct
  REGION 1..540: note = synthetic_tcPanD (wild)
MPATGEDQDLVQDLIEEPATFSDAVLSSDEELFHQKCPKPAPIYSPVSKPVSFESLPNRRLHEEFLRSSVDVLLQEAVFEGTNRKNRVLQWREPEELRRLMDFGVRSAPSTHEELLEVLKKVVTYSVKTGHPYFVNQLFSAVDPYGLVAQWATDALNPSVYTYEVSPVFVLMEEVVLREMRAIVGFEGGKGDGIFCPGGSIANGYAISCARYRFMPDIKKKGLHSLPRLVLFTSEDAHYSIKKLASFQGIGTDNVYLIRTDARGRMDVSHLVEEIERSLREGAAPFMVSATAGTTVIGAFDPIEKIADVCQKYKLWLHVDAAWGGGALVSAKHRHLLKGIERADSVTWNPHKLLTAPQQCSTLLLRHEGVLAEAHSTNAAYLFQKDKFYDTKYDTGDKHIQCGRRADVLKFWFMWKAKGTSGLEKHVDKVFENARFFTDCIKNREGFEMVIAEPEYTNICFWYVPKSLRGRKDEADYKDKLHKVAPRIKERMMKEGSMMVTYQAQKGHPNFFRIVFQNSGLDKADMVHLVEEIERLGSDL

SEQ ID NO: 52 - protein, 540 aa, synthetic construct
  REGION 1..540: note = synthetic_tcPanD F139Y (var.)
MPATGEDQDLVQDLIEEPATFSDAVLSSDEELFHQKCPKPAPIYSPVSKPVSFESLPNRRLHEEFLRSSVDVLLQEAVFEGTNRKNRVLQWREPEELRRLMDFGVRSAPSTHEELLEVLKKVVTYSVKTGHPYFVNQLYSAVDPYGLVAQWATDALNPSVYTYEVSPVFVLMEEVVLREMRAIVGFEGGKGDGIFCPGGSIANGYAISCARYRFMPDIKKKGLHSLPRLVLFTSEDAHYSIKKLASFQGIGTDNVYLIRTDARGRMDVSHLVEEIERSLREGAAPFMVSATAGTTVIGAFDPIEKIADVCQKYKLWLHVDAAWGGGALVSAKHRHLLKGIERADSVTWNPHKLLTAPQQCSTLLLRHEGVLAEAHSTNAAYLFQKDKFYDTKYDTGDKHIQCGRRADVLKFWFMWKAKGTSGLEKHVDKVFENARFFTDCIKNREGFEMVIAEPEYTNICFWYVPKSLRGRKDEADYKDKLHKVAPRIKERMMKEGSMMVTYQAQKGHPNFFRIVFQNSGLDKADMVHLVEEIERLGSDL

SEQ ID NO: 53 - protein, 540 aa, synthetic construct
  REGION 1..540: note = synthetic_tcPanD F139T (var.)
MPATGEDQDLVQDLIEEPATFSDAVLSSDEELFHQKCPKPAPIYSPVSKPVSFESLPNRRLHEEFLRSSVDVLLQEAVFEGTNRKNRVLQWREPEELRRLMDFGVRSAPSTHEELLEVLKKVVTYSVKTGHPYFVNQLTSAVDPYGLVAQWATDALNPSVYTYEVSPVFVLMEEVVLREMRAIVGFEGGKGDGIFCPGGSIANGYAISCARYRFMPDIKKKGLHSLPRLVLFTSEDAHYSIKKLASFQGIGTDNVYLIRTDARGRMDVSHLVEEIERSLREGAAPFMVSATAGTTVIGAFDPIEKIADVCQKYKLWLHVDAAWGGGALVSAKHRHLLKGIERADSVTWNPHKLLTAPQQCSTLLLRHEGVLAEAHSTNAAYLFQKDKFYDTKYDTGDKHIQCGRRADVLKFWFMWKAKGTSGLEKHVDKVFENARFFTDCIKNREGFEMVIAEPEYTNICFWYVPKSLRGRKDEADYKDKLHKVAPRIKERMMKEGSMMVTYQAQKGHPNFFRIVFQNSGLDKADMVHLVEEIERLGSDL

SEQ ID NO: 54 - protein, 540 aa, synthetic construct
  REGION 1..540: note = synthetic_tcPanD F139A (var.)
MPATGEDQDLVQDLIEEPATFSDAVLSSDEELFHQKCPKPAPIYSPVSKPVSFESLPNRRLHEEFLRSSVDVLLQEAVFEGTNRKNRVLQWREPEELRRLMDFGVRSAPSTHEELLEVLKKVVTYSVKTGHPYFVNQLASAVDPYGLVAQWATDALNPSVYTYEVSPVFVLMEEVVLREMRAIVGFEGGKGDGIFCPGGSIANGYAISCARYRFMPDIKKKGLHSLPRLVLFTSEDAHYSIKKLASFQGIGTDNVYLIRTDARGRMDVSHLVEEIERSLREGAAPFMVSATAGTTVIGAFDPIEKIADVCQKYKLWLHVDAAWGGGALVSAKHRHLLKGIERADSVTWNPHKLLTAPQQCSTLLLRHEGVLAEAHSTNAAYLFQKDKFYDTKYDTGDKHIQCGRRADVLKFWFMWKAKGTSGLEKHVDKVFENARFFTDCIKNREGFEMVIAEPEYTNICFWYVPKSLRGRKDEADYKDKLHKVAPRIKERMMKEGSMMVTYQAQKGHPNFFRIVFQNSGLDKADMVHLVEEIERLGSDL

SEQ ID NO: 55 - protein, 540 aa, synthetic construct
  REGION 1..540: note = synthetic_tcPanD F139S (var.)
MPATGEDQDLVQDLIEEPATFSDAVLSSDEELFHQKCPKPAPIYSPVSKPVSFESLPNRRLHEEFLRSSVDVLLQEAVFEGTNRKNRVLQWREPEELRRLMDFGVRSAPSTHEELLEVLKKVVTYSVKTGHPYFVNQLSSAVDPYGLVAQWATDALNPSVYTYEVSPVFVLMEEVVLREMRAIVGFEGGKGDGIFCPGGSIANGYAISCARYRFMPDIKKKGLHSLPRLVLFTSEDAHYSIKKLASFQGIGTDNVYLIRTDARGRMDVSHLVEEIERSLREGAAPFMVSATAGTTVIGAFDPIEKIADVCQKYKLWLHVDAAWGGGALVSAKHRHLLKGIERADSVTWNPHKLLTAPQQCSTLLLRHEGVLAEAHSTNAAYLFQKDKFYDTKYDTGDKHIQCGRRADVLKFWFMWKAKGTSGLEKHVDKVFENARFFTDCIKNREGFEMVIAEPEYTNICFWYVPKSLRGRKDEADYKDKLHKVAPRIKERMMKEGSMMVTYQAQKGHPNFFRIVFQNSGLDKADMVHLVEEIERLGSDL

SEQ ID NO: 56 - protein, 540 aa, synthetic construct
  REGION 1..540: note = synthetic_tcPanD F139L (var.)
MPATGEDQDLVQDLIEEPATFSDAVLSSDEELFHQKCPKPAPIYSPVSKPVSFESLPNRRLHEEFLRSSVDVLLQEAVFEGTNRKNRVLQWREPEELRRLMDFGVRSAPSTHEELLEVLKKVVTYSVKTGHPYFVNQLLSAVDPYGLVAQWATDALNPSVYTYEVSPVFVLMEEVVLREMRAIVGFEGGKGDGIFCPGGSIANGYAISCARYRFMPDIKKKGLHSLPRLVLFTSEDAHYSIKKLASFQGIGTDNVYLIRTDARGRMDVSHLVEEIERSLREGAAPFMVSATAGTTVIGAFDPIEKIADVCQKYKLWLHVDAAWGGGALVSAKHRHLLKGIERADSVTWNPHKLLTAPQQCSTLLLRHEGVLAEAHSTNAAYLFQKDKFYDTKYDTGDKHIQCGRRADVLKFWFMWKAKGTSGLEKHVDKVFENARFFTDCIKNREGFEMVIAEPEYTNICFWYVPKSLRGRKDEADYKDKLHKVAPRIKERMMKEGSMMVTYQAQKGHPNFFRIVFQNSGLDKADMVHLVEEIERLGSDL

SEQ ID NO: 57 - protein, 540 aa, synthetic construct
  REGION 1..540: note = synthetic_tcPanD F139I (var.)
MPATGEDQDLVQDLIEEPATFSDAVLSSDEELFHQKCPKPAPIYSPVSKPVSFESLPNRRLHEEFLRSSVDVLLQEAVFEGTNRKNRVLQWREPEELRRLMDFGVRSAPSTHEELLEVLKKVVTYSVKTGHPYFVNQLISAVDPYGLVAQWATDALNPSVYTYEVSPVFVLMEEVVLREMRAIVGFEGGKGDGIFCPGGSIANGYAISCARYRFMPDIKKKGLHSLPRLVLFTSEDAHYSIKKLASFQGIGTDNVYLIRTDARGRMDVSHLVEEIERSLREGAAPFMVSATAGTTVIGAFDPIEKIADVCQKYKLWLHVDAAWGGGALVSAKHRHLLKGIERADSVTWNPHKLLTAPQQCSTLLLRHEGVLAEAHSTNAAYLFQKDKFYDTKYDTGDKHIQCGRRADVLKFWFMWKAKGTSGLEKHVDKVFENARFFTDCIKNREGFEMVIAEPEYTNICFWYVPKSLRGRKDEADYKDKLHKVAPRIKERMMKEGSMMVTYQAQKGHPNFFRIVFQNSGLDKADMVHLVEEIERLGSDL

SEQ ID NO: 58 - protein, 540 aa, synthetic construct
  REGION 1..540: note = synthetic_tcPanD F139V (var.)
MPATGEDQDLVQDLIEEPATFSDAVLSSDEELFHQKCPKPAPIYSPVSKPVSFESLPNRRLHEEFLRSSVDVLLQEAVFEGTNRKNRVLQWREPEELRRLMDFGVRSAPSTHEELLEVLKKVVTYSVKTGHPYFVNQLVSAVDPYGLVAQWATDALNPSVYTYEVSPVFVLMEEVVLREMRAIVGFEGGKGDGIFCPGGSIANGYAISCARYRFMPDIKKKGLHSLPRLVLFTSEDAHYSIKKLASFQGIGTDNVYLIRTDARGRMDVSHLVEEIERSLREGAAPFMVSATAGTTVIGAFDPIEKIADVCQKYKLWLHVDAAWGGGALVSAKHRHLLKGIERADSVTWNPHKLLTAPQQCSTLLLRHEGVLAEAHSTNAAYLFQKDKFYDTKYDTGDKHIQCGRRADVLKFWFMWKAKGTSGLEKHVDKVFENARFFTDCIKNREGFEMVIAEPEYTNICFWYVPKSLRGRKDEADYKDKLHKVAPRIKERMMKEGSMMVTYQAQKGHPNFFRIVFQNSGLDKADMVHLVEEIERLGSDL

SEQ ID NO: 59 - protein, 540 aa, synthetic construct
  REGION 1..540: note = synthetic_tcPanD F139D (var.)
MPATGEDQDLVQDLIEEPATFSDAVLSSDEELFHQKCPKPAPIYSPVSKPVSFESLPNRRLHEEFLRSSVDVLLQEAVFEGTNRKNRVLQWREPEELRRLMDFGVRSAPSTHEELLEVLKKVVTYSVKTGHPYFVNQLDSAVDPYGLVAQWATDALNPSVYTYEVSPVFVLMEEVVLREMRAIVGFEGGKGDGIFCPGGSIANGYAISCARYRFMPDIKKKGLHSLPRLVLFTSEDAHYSIKKLASFQGIGTDNVYLIRTDARGRMDVSHLVEEIERSLREGAAPFMVSATAGTTVIGAFDPIEKIADVCQKYKLWLHVDAAWGGGALVSAKHRHLLKGIERADSVTWNPHKLLTAPQQCSTLLLRHEGVLAEAHSTNAAYLFQKDKFYDTKYDTGDKHIQCGRRADVLKFWFMWKAKGTSGLEKHVDKVFENARFFTDCIKNREGFEMVIAEPEYTNICFWYVPKSLRGRKDEADYKDKLHKVAPRIKERMMKEGSMMVTYQAQKGHPNFFRIVFQNSGLDKADMVHLVEEIERLGSDL

SEQ ID NO: 60 - protein, 540 aa, synthetic construct
  REGION 1..540: note = synthetic_tcPanD F139G (var.)
MPATGEDQDLVQDLIEEPATFSDAVLSSDEELFHQKCPKPAPIYSPVSKPVSFESLPNRRLHEEFLRSSVDVLLQEAVFEGTNRKNRVLQWREPEELRRLMDFGVRSAPSTHEELLEVLKKVVTYSVKTGHPYFVNQLGSAVDPYGLVAQWATDALNPSVYTYEVSPVFVLMEEVVLREMRAIVGFEGGKGDGIFCPGGSIANGYAISCARYRFMPDIKKKGLHSLPRLVLFTSEDAHYSIKKLASFQGIGTDNVYLIRTDARGRMDVSHLVEEIERSLREGAAPFMVSATAGTTVIGAFDPIEKIADVCQKYKLWLHVDAAWGGGALVSAKHRHLLKGIERADSVTWNPHKLLTAPQQCSTLLLRHEGVLAEAHSTNAAYLFQKDKFYDTKYDTGDKHIQCGRRADVLKFWFMWKAKGTSGLEKHVDKVFENARFFTDCIKNREGFEMVIAEPEYTNICFWYVPKSLRGRKDEADYKDKLHKVAPRIKERMMKEGSMMVTYQAQKGHPNFFRIVFQNSGLDKADMVHLVEEIERLGSDL

SEQ ID NO: 61 - protein, 540 aa, synthetic construct
  REGION 1..540: note = synthetic_tcPanD F139H (var.)
MPATGEDQDLVQDLIEEPATFSDAVLSSDEELFHQKCPKPAPIYSPVSKPVSFESLPNRRLHEEFLRSSVDVLLQEAVFEGTNRKNRVLQWREPEELRRLMDFGVRSAPSTHEELLEVLKKVVTYSVKTGHPYFVNQLHSAVDPYGLVAQWATDALNPSVYTYEVSPVFVLMEEVVLREMRAIVGFEGGKGDGIFCPGGSIANGYAISCARYRFMPDIKKKGLHSLPRLVLFTSEDAHYSIKKLASFQGIGTDNVYLIRTDARGRMDVSHLVEEIERSLREGAAPFMVSATAGTTVIGAFDPIEKIADVCQKYKLWLHVDAAWGGGALVSAKHRHLLKGIERADSVTWNPHKLLTAPQQCSTLLLRHEGVLAEAHSTNAAYLFQKDKFYDTKYDTGDKHIQCGRRADVLKFWFMWKAKGTSGLEKHVDKVFENARFFTDCIKNREGFEMVIAEPEYTNICFWYVPKSLRGRKDEADYKDKLHKVAPRIKERMMKEGSMMVTYQAQKGHPNFFRIVFQNSGLDKADMVHLVEEIERLGSDL

SEQ ID NO: 62 - DNA, 1623 bp, synthetic construct
  misc_feature 1..1623: note = synthetic_gene coding tcPanD (wild)
  source 1..1623: mol_type = other DNA
atgccggcaaccggagaggaccaagacttggttcaggacttgatcgaggaacctgccactttcagcgacgctgtgttgtcctccgacgaggaactgtttcaccagaaatgcccgaagccggcaccaatttactcgccagtgtcaaaacccgtttcattcgagagcctgcccaatcgccgccttcatgaagaatttctccgctcatcggttgatgtactcctgcaggaggccgttttcgagggaactaatcggaagaatcgggtgcttcagtggcgtgagccagaggaattgcggcgtctcatggattttggcgttcggtctgctccttcaacccacgaagaactgctggaagttcttaaaaaagtagtcacgtacagcgtcaagaccggccacccctactttgtaaatcaactcttcagcgctgtcgacccctatggcctggtcgcgcaatgggctaccgatgccttgaatccctcagtgtacacgtacgaagttagcccggtcttcgtccttatggaggaagtcgtcctgcgtgaaatgcgtgcgattgtcggctttgagggaggcaagggagacggaattttctgtccaggtggctctatcgccaacggttacgcaatttcgtgtgcacggtatcgtttcatgccggatattaagaaaaaaggactgcactcacttccacggctggtactcttcacctcggaagacgctcactactcgatcaaaaaactggcatccttccagggcatcggcaccgataacgtttaccttatccgtactgatgcacggggccggatggatgtttctcacctggtggaggaaattgagcgctcgttgcgtgagggtgccgccccgttcatggtatccgccaccgcaggtacgacggtgatcggagcttttgaccctatcgaaaagatcgccgatgtctgccagaaatacaaattgtggctccacgttgacgctgcctggggtggaggagccttggtctcggctaagcatcgccatctgctcaaaggcatcgagcgggctgattctgttacgtggaatcctcataaactgcttaccgcaccccaacagtgcagcactttgcttcttcgccatgaaggcgtactggcggaagcacatagcaccaatgctgcttacctgttccagaaggacaagttttacgacaccaaatacgacaccggcgataaacacatccaatgtggtcggcgtgccgacgtgttgaaattctggttcatgtggaaggctaaaggcacctccggcttggaaaaacacgttgataaggtatttgaaaacgctcggttctttaccgactgtattaaaaaccgtgagggattcgagatggtaattgctgagccagagtatacgaacatctgtttctggtacgtaccaaaatccctgcggggccggaaggatgaagctgattataaagacaaattgcataaagtcgctccacgtatcaaggaacgcatgatgaaagagggctcgatgatggttacgtaccaggcacagaagggccacccgaattttttccgtattgtgttccaaaatagcggactcgataaagctgatatggtccaccttgtcgaagagatcgaacggcttggttcagatttgtaa

SEQ ID NO: 63 - DNA, 1623 bp, synthetic construct
  misc_feature 1..1623: note = synthetic_gene coding tcPanD F139Y (var.)
  source 1..1623: mol_type = other DNA
atgccggcaaccggagaggaccaagacttggttcaggacttgatcgaggaacctgccactttcagcgacgctgtgttgtcctccgacgaggaactgtttcaccagaaatgcccgaagccggcaccaatttactcgccagtgtcaaaacccgtttcattcgagagcctgcccaatcgccgccttcatgaagaatttctccgctcatcggttgatgtactcctgcaggaggccgttttcgagggaactaatcggaagaatcgggtgcttcagtggcgtgagccagaggaattgcggcgtctcatggattttggcgttcggtctgctccttcaacccacgaagaactgctggaagttcttaaaaaagtagtcacgtacagcgtcaagaccggccacccctactttgtaaatcaactctacagcgctgtcgacccctatggcctggtcgcgcaatgggctaccgatgccttgaatccctcagtgtacacgtacgaagttagcccggtcttcgtccttatggaggaagtcgtcctgcgtgaaatgcgtgcgattgtcggctttgagggaggcaagggagacggaattttctgtccaggtggctctatcgccaacggttacgcaatttcgtgtgcacggtatcgtttcatgccggatattaagaaaaaaggactgcactcacttccacggctggtactcttcacctcggaagacgctcactactcgatcaaaaaactggcatccttccagggcatcggcaccgataacgtttaccttatccgtactgatgcacggggccggatggatgtttctcacctggtggaggaaattgagcgctcgttgcgtgagggtgccgccccgttcatggtatccgccaccgcaggtacgacggtgatcggagcttttgaccctatcgaaaagatcgccgatgtctgccagaaatacaaattgtggctccacgttgacgctgcctggggtggaggagccttggtctcggctaagcatcgccatctgctcaaaggcatcgagcgggctgattctgttacgtggaatcctcataaactgcttaccgcaccccaacagtgcagcactttgcttcttcgccatgaaggcgtactggcggaagcacatagcaccaatgctgcttacctgttccagaaggacaagttttacgacaccaaatacgacaccggcgataaacacatccaatgtggtcggcgtgccgacgtgttgaaattctggttcatgtggaaggctaaaggcacctccggcttggaaaaacacgttgataaggtatttgaaaacgctcggttctttaccgactgtattaaaaaccgtgagggattcgagatggtaattgctgagccagagtatacgaacatctgtttctggtacgtaccaaaatccctgcggggccggaaggatgaagctgattataaagacaaattgcataaagtcgctccacgtatcaaggaacgcatgatgaaagagggctcgatgatggttacgtaccaggcacagaagggccacccgaattttttccgtattgtgttccaaaatagcggactcgataaagctgatatggtccaccttgtcgaagagatcgaacggcttggttcagatttgtaa

SEQ ID NO: 64 - DNA, 1623 bp, synthetic construct
  misc_feature 1..1623: note = synthetic_gene coding tcPanD F139T (var.)
  source 1..1623: mol_type = other DNA
atgccggcaaccggagaggaccaagacttggttcaggacttgatcgaggaacctgccactttcagcgacgctgtgttgtcctccgacgaggaactgtttcaccagaaatgcccgaagccggcaccaatttactcgccagtgtcaaaacccgtttcattcgagagcctgcccaatcgccgccttcatgaagaatttctccgctcatcggttgatgtactcctgcaggaggccgttttcgagggaactaatcggaagaatcgggtgcttcagtggcgtgagccagaggaattgcggcgtctcatggattttggcgttcggtctgctccttcaacccacgaagaactgctggaagttcttaaaaaagtagtcacgtacagcgtcaagaccggccacccctactttgtaaatcaactcaccagcgctgtcgacccctatggcctggtcgcgcaatgggctaccgatgccttgaatccctcagtgtacacgtacgaagttagcccggtcttcgtccttatggaggaagtcgtcctgcgtgaaatgcgtgcgattgtcggctttgagggaggcaagggagacggaattttctgtccaggtggctctatcgccaacggttacgcaatttcgtgtgcacggtatcgtttcatgccggatattaagaaaaaaggactgcactcacttccacggctggtactcttcacctcggaagacgctcactactcgatcaaaaaactggcatccttccagggcatcggcaccgataacgtttaccttatccgtactgatgcacggggccggatggatgtttctcacctggtggaggaaattgagcgctcgttgcgtgagggtgccgccccgttcatggtatccgccaccgcaggtacgacggtgatcggagcttttgaccctatcgaaaagatcgccgatgtctgccagaaatacaaattgtggctccacgttgacgctgcctggggtggaggagccttggtctcggctaagcatcgccatctgctcaaaggcatcgagcgggctgattctgttacgtggaatcctcataaactgcttaccgcaccccaacagtgcagcactttgcttcttcgccatgaaggcgtactggcggaagcacatagcaccaatgctgcttacctgttccagaaggacaagttttacgacaccaaatacgacaccggcgataaacacatccaatgtggtcggcgtgccgacgtgttgaaattctggttcatgtggaaggctaaaggcacctccggcttggaaaaacacgttgataaggtatttgaaaacgctcggttctttaccgactgtattaaaaaccgtgagggattcgagatggtaattgctgagccagagtatacgaacatctgtttctggtacgtaccaaaatccctgcggggccggaaggatgaagctgattataaagacaaattgcataaagtcgctccacgtatcaaggaacgcatgatgaaagagggctcgatgatggttacgtaccaggcacagaagggccacccgaattttttccgtattgtgttccaaaatagcggactcgataaagctgatatggtccaccttgtcgaagagatcgaacggcttggttcagatttgtaa

SEQ ID NO: 65 - DNA, 1623 bp, synthetic construct
  misc_feature 1..1623: note = synthetic_gene coding tcPanD F139A (var.)
  source 1..1623: mol_type = other DNA
atgccggcaaccggagaggaccaagacttggttcaggacttgatcgaggaacctgccactttcagcgacgctgtgttgtcctccgacgaggaactgtttcaccagaaatgcccgaagccggcaccaatttactcgccagtgtcaaaacccgtttcattcgagagcctgcccaatcgccgccttcatgaagaatttctccgctcatcggttgatgtactcctgcaggaggccgttttcgagggaactaatcggaagaatcgggtgcttcagtggcgtgagccagaggaattgcggcgtctcatggattttggcgttcggtctgctccttcaacccacgaagaactgctggaagttcttaaaaaagtagtcacgtacagcgtcaagaccggccacccctactttgtaaatcaactcgctagcgctgtcgacccctatggcctggtcgcgcaatgggctaccgatgccttgaatccctcagtgtacacgtacgaagttagcccggtcttcgtccttatggaggaagtcgtcctgcgtgaaatgcgtgcgattgtcggctttgagggaggcaagggagacggaattttctgtccaggtggctctatcgccaacggttacgcaatttcgtgtgcacggtatcgtttcatgccggatattaagaaaaaaggactgcactcacttccacggctggtactcttcacctcggaagacgctcactactcgatcaaaaaactggcatccttccagggcatcggcaccgataacgtttaccttatccgtactgatgcacggggccggatggatgtttctcacctggtggaggaaattgagcgctcgttgcgtgagggtgccgccccgttcatggtatccgccaccgcaggtacgacggtgatcggagcttttgaccctatcgaaaagatcgccgatgtctgccagaaatacaaattgtggctccacgttgacgctgcctggggtggaggagccttggtctcggctaagcatcgccatctgctcaaaggcatcgagcgggctgattctgttacgtggaatcctcataaactgcttaccgcaccccaacagtgcagcactttgcttcttcgccatgaaggcgtactggcggaagcacatagcaccaatgctgcttacctgttccagaaggacaagttttacgacaccaaatacgacaccggcgataaacacatccaatgtggtcggcgtgccgacgtgttgaaattctggttcatgtggaaggctaaaggcacctccggcttggaaaaacacgttgataaggtatttgaaaacgctcggttctttaccgactgtattaaaaaccgtgagggattcgagatggtaattgctgagccagagtatacgaacatctgtttctggtacgtaccaaaatccctgcggggccggaaggatgaagctgattataaagacaaattgcataaagtcgctccacgtatcaaggaacgcatgatgaaagagggctcgatgatggttacgtaccaggcacagaagggccacccgaattttttccgtattgtgttccaaaatagcggactcgataaagctgatatggtccaccttgtcgaagagatcgaacggcttggttcagatttgtaa

SEQ ID NO: 66 - DNA, 1623 bp, synthetic construct
  misc_feature 1..1623: note = synthetic_gene coding tcPanD F139S (var.)
  source 1..1623: mol_type = other DNA
atgccggcaaccggagaggaccaagacttggttcaggacttgatcgaggaacctgccactttcagcgacgctgtgttgtcctccgacgaggaactgtttcaccagaaatgcccgaagccggcaccaatttactcgccagtgtcaaaacccgtttcattcgagagcctgcccaatcgccgccttcatgaagaatttctccgctcatcggttgatgtactcctgcaggaggccgttttcgagggaactaatcggaagaatcgggtgcttcagtggcgtgagccagaggaattgcggcgtctcatggattttggcgttcggtctgctccttcaacccacgaagaactgctggaagttcttaaaaaagtagtcacgtacagcgtcaagaccggccacccctactttgtaaatcaactctctagcgctgtcgacccctatggcctggtcgcgcaatgggctaccgatgccttgaatccctcagtgtacacgtacgaagttagcccggtcttcgtccttatggaggaagtcgtcctgcgtgaaatgcgtgcgattgtcggctttgagggaggcaagggagacggaattttctgtccaggtggctctatcgccaacggttacgcaatttcgtgtgcacggtatcgtttcatgccggatattaagaaaaaaggactgcactcacttccacggctggtactcttcacctcggaagacgctcactactcgatcaaaaaactggcatccttccagggcatcggcaccgataacgtttaccttatccgtactgatgcacggggccggatggatgtttctcacctggtggaggaaattgagcgctcgttgcgtgagggtgccgccccgttcatggtatccgccaccgcaggtacgacggtgatcggagcttttgaccctatcgaaaagatcgccgatgtctgccagaaatacaaattgtggctccacgttgacgctgcctggggtggaggagccttggtctcggctaagcatcgccatctgctcaaaggcatcgagcgggctgattctgttacgtggaatcctcataaactgcttaccgcaccccaacagtgcagcactttgcttcttcgccatgaaggcgtactggcggaagcacatagcaccaatgctgcttacctgttccagaaggacaagttttacgacaccaaatacgacaccggcgataaacacatccaatgtggtcggcgtgccgacgtgttgaaattctggttcatgtggaaggctaaaggcacctccggcttggaaaaacacgttgataaggtatttgaaaacgctcggttctttaccgactgtattaaaaaccgtgagggattcgagatggtaattgctgagccagagtatacgaacatctgtttctggtacgtaccaaaatccctgcggggccggaaggatgaagctgattataaagacaaattgcataaagtcgctccacgtatcaaggaacgcatgatgaaagagggctcgatgatggttacgtaccaggcacagaagggccacccgaattttttccgtattgtgttccaaaatagcggactcgataaagctgatatggtccaccttgtcgaagagatcgaacggcttggttcagatttgtaa

SEQ ID NO: 67 - DNA, 1623 bp, synthetic construct
  misc_feature 1..1623: note = synthetic_gene coding tcPanD F139L (var.)
  source 1..1623: mol_type = other DNA
atgccggcaaccggagaggaccaagacttggttcaggacttgatcgaggaacctgccactttcagcgacgctgtgttgtcctccgacgaggaactgtttcaccagaaatgcccgaagccggcaccaatttactcgccagtgtcaaaacccgtttcattcgagagcctgcccaatcgccgccttcatgaagaatttctccgctcatcggttgatgtactcctgcaggaggccgttttcgagggaactaatcggaagaatcgggtgcttcagtggcgtgagccagaggaattgcggcgtctcatggattttggcgttcggtctgctccttcaacccacgaagaactgctggaagttcttaaaaaagtagtcacgtacagcgtcaagaccggccacccctactttgtaaatcaactccttagcgctgtcgacccctatggcctggtcgcgcaatgggctaccgatgccttgaatccctcagtgtacacgtacgaagttagcccggtcttcgtccttatggaggaagtcgtcctgcgtgaaatgcgtgcgattgtcggctttgagggaggcaagggagacggaattttctgtccaggtggctctatcgccaacggttacgcaatttcgtgtgcacggtatcgtttcatgccggatattaagaaaaaaggactgcactcacttccacggctggtactcttcacctcggaagacgctcactactcgatcaaaaaactggcatccttccagggcatcggcaccgataacgtttaccttatccgtactgatgcacggggccggatggatgtttctcacctggtggaggaaattgagcgctcgttgcgtgagggtgccgccccgttcatggtatccgccaccgcaggtacgacggtgatcggagcttttgaccctatcgaaaagatcgccgatgtctgccagaaatacaaattgtggctccacgttgacgctgcctggggtggaggagccttggtctcggctaagcatcgccatctgctcaaaggcatcgagcgggctgattctgttacgtggaatcctcataaactgcttaccgcaccccaacagtgcagcactttgcttcttcgccatgaaggcgtactggcggaagcacatagcaccaatgctgcttacctgttccagaaggacaagttttacgacaccaaatacgacaccggcgataaacacatccaatgtggtcggcgtgccgacgtgttgaaattctggttcatgtggaaggctaaaggcacctccggcttggaaaaacacgttgataaggtatttgaaaacgctcggttctttaccgactgtattaaaaaccgtgagggattcgagatggtaattgctgagccagagtatacgaacatctgtttctggtacgtaccaaaatccctgcggggccggaaggatgaagctgattataaagacaaattgcataaagtcgctccacgtatcaaggaacgcatgatgaaagagggctcgatgatggttacgtaccaggcacagaagggccacccgaattttttccgtattgtgttccaaaatagcggactcgataaagctgatatggtccaccttgtcgaagagatcgaacggcttggttcagatttgtaa

SEQ ID NO: 68 - DNA, 1623 bp, synthetic construct
  misc_feature 1..1623: note = synthetic_gene coding tcPanD F139I (var.)
  source 1..1623: mol_type = other DNA
atgccggcaaccggagaggaccaagacttggttcaggacttgatcgaggaacctgccactttcagcgacgctgtgttgtcctccgacgaggaactgtttcaccagaaatgcccgaagccggcaccaatttactcgccagtgtcaaaacccgtttcattcgagagcctgcccaatcgccgccttcatgaagaatttctccgctcatcggttgatgtactcctgcaggaggccgttttcgagggaactaatcggaagaatcgggtgcttcagtggcgtgagccagaggaattgcggcgtctcatggattttggcgttcggtctgctccttcaacccacgaagaactgctggaagttcttaaaaaagtagtcacgtacagcgtcaagaccggccacccctactttgtaaatcaactcatcagcgctgtcgacccctatggcctggtcgcgcaatgggctaccgatgccttgaatccctcagtgtacacgtacgaagttagcccggtcttcgtccttatggaggaagtcgtcctgcgtgaaatgcgtgcgattgtcggctttgagggaggcaagggagacggaattttctgtccaggtggctctatcgccaacggttacgcaatttcgtgtgcacggtatcgtttcatgccggatattaagaaaaaaggactgcactcacttccacggctggtactcttcacctcggaagacgctcactactcgatcaaaaaactggcatccttccagggcatcggcaccgataacgtttaccttatccgtactgatgcacggggccggatggatgtttctcacctggtggaggaaattgagcgctcgttgcgtgagggtgccgccccgttcatggtatccgccaccgcaggtacgacggtgatcggagcttttgaccctatcgaaaagatcgccgatgtctgccagaaatacaaattgtggctccacgttgacgctgcctggggtggaggagccttggtctcggctaagcatcgccatctgctcaaaggcatcgagcgggctgattctgttacgtggaatcctcataaactgcttaccgcaccccaacagtgcagcactttgcttcttcgccatgaaggcgtactggcggaagcacatagcaccaatgctgcttacctgttccagaaggacaagttttacgacaccaaatacgacaccggcgataaacacatccaatgtggtcggcgtgccgacgtgttgaaattctggttcatgtggaaggctaaaggcacctccggcttggaaaaacacgttgataaggtatttgaaaacgctcggttctttaccgactgtattaaaaaccgtgagggattcgagatggtaattgctgagccagagtatacgaacatctgtttctggtacgtaccaaaatccctgcggggccggaaggatgaagctgattataaagacaaattgcataaagtcgctccacgtatcaaggaacgcatgatgaaagagggctcgatgatggttacgtaccaggcacagaagggccacccgaattttttccgtattgtgttccaaaatagcggactcgataaagctgatatggtccaccttgtcgaagagatcgaacggcttggttcagatttgtaa

SEQ ID NO: 69 - DNA, 1623 bp, synthetic construct
  misc_feature 1..1623: note = synthetic_gene coding tcPanD F139V (var.)
  source 1..1623: mol_type = other DNA
atgccggcaaccggagaggaccaagacttggttcaggacttgatcgaggaacctgccactttcagcgacgctgtgttgtcctccgacgaggaactgtttcaccagaaatgcccgaagccggcaccaatttactcgccagtgtcaaaacccgtttcattcgagagcctgcccaatcgccgccttcatgaagaatttctccgctcatcggttgatgtactcctgcaggaggccgttttcgagggaactaatcggaagaatcgggtgcttcagtggcgtgagccagaggaattgcggcgtctcatggattttggcgttcggtctgctccttcaacccacgaagaactgctggaagttcttaaaaaagtagtcacgtacagcgtcaagaccggccacccctactttgtaaatcaactcgtgagcgctgtcgacccctatggcctggtcgcgcaatgggctaccgatgccttgaatccctcagtgtacacgtacgaagttagcccggtcttcgtccttatggaggaagtcgtcctgcgtgaaatgcgtgcgattgtcggctttgagggaggcaagggagacggaattttctgtccaggtggctctatcgccaacggttacgcaatttcgtgtgcacggtatcgtttcatgccggatattaagaaaaaaggactgcactcacttccacggctggtactcttcacctcggaagacgctcactactcgatcaaaaaactggcatccttccagggcatcggcaccgataacgtttaccttatccgtactgatgcacggggccggatggatgtttctcacctggtggaggaaattgagcgctcgttgcgtgagggtgccgccccgttcatggtatccgccaccgcaggtacgacggtgatcggagcttttgaccctatcgaaaagatcgccgatgtctgccagaaatacaaattgtggctccacgttgacgctgcctggggtggaggagccttggtctcggctaagcatcgccatctgctcaaaggcatcgagcgggctgattctgttacgtggaatcctcataaactgcttaccgcaccccaacagtgcagcactttgcttcttcgccatgaaggcgtactggcggaagcacatagcaccaatgctgcttacctgttccagaaggacaagttttacgacaccaaatacgacaccggcgataaacacatccaatgtggtcggcgtgccgacgtgttgaaattctggttcatgtggaaggctaaaggcacctccggcttggaaaaacacgttgataaggtatttgaaaacgctcggttctttaccgactgtattaaaaaccgtgagggattcgagatggtaattgctgagccagagtatacgaacatctgtttctggtacgtaccaaaatccctgcggggccggaaggatgaagctgattataaagacaaattgcataaagtcgctccacgtatcaaggaacgcatgatgaaagagggctcgatgatggttacgtaccaggcacagaagggccacccgaattttttccgtattgtgttccaaaatagcggactcgataaagctgatatggtccaccttgtcgaagagatcgaacggcttggttcagatttgtaa

SEQ ID NO: 70 - DNA, 1623 bp, synthetic construct
  misc_feature 1..1623: note = synthetic_gene coding tcPanD F139D (var.)
  source 1..1623: mol_type = other DNA
atgccggcaaccggagaggaccaagacttggttcaggacttgatcgaggaacctgccactttcagcgacgctgtgttgtcctccgacgaggaactgtttcaccagaaatgcccgaagccggcaccaatttactcgccagtgtcaaaacccgtttcattcgagagcctgcccaatcgccgccttcatgaagaatttctccgctcatcggttgatgtactcctgcaggaggccgttttcgagggaactaatcggaagaatcgggtgcttcagtggcgtgagccagaggaattgcggcgtctcatggattttggcgttcggtctgctccttcaacccacgaagaactgctggaagttcttaaaaaagtagtcacgtacagcgtcaagaccggccacccctactttgtaaatcaactcgatagcgctgtcgacccctatggcctggtcgcgcaatgggctaccgatgccttgaatccctcagtgtacacgtacgaagttagcccggtcttcgtccttatggaggaagtcgtcctgcgtgaaatgcgtgcgattgtcggctttgagggaggcaagggagacggaattttctgtccaggtggctctatcgccaacggttacgcaatttcgtgtgcacggtatcgtttcatgccggatattaagaaaaaaggactgcactcacttccacggctggtactcttcacctcggaagacgctcactactcgatcaaaaaactggcatccttccagggcatcggcaccgataacgtttaccttatccgtactgatgcacggggccggatggatgtttctcacctggtggaggaaattgagcgctcgttgcgtgagggtgccgccccgttcatggtatccgccaccgcaggtacgacggtgatcggagcttttgaccctatcgaaaagatcgccgatgtctgccagaaatacaaattgtggctccacgttgacgctgcctggggtggaggagccttggtctcggctaagcatcgccatctgctcaaaggcatcgagcgggctgattctgttacgtggaatcctcataaactgcttaccgcaccccaacagtgcagcactttgcttcttcgccatgaaggcgtactggcggaagcacatagcaccaatgctgcttacctgttccagaaggacaagttttacgacaccaaatacgacaccggcgataaacacatccaatgtggtcggcgtgccgacgtgttgaaattctggttcatgtggaaggctaaaggcacctccggcttggaaaaacacgttgataaggtatttgaaaacgctcggttctttaccgactgtattaaaaaccgtgagggattcgagatggtaattgctgagccagagtatacgaacatctgtttctggtacgtaccaaaatccctgcggggccggaaggatgaagctgattataaagacaaattgcataaagtcgctccacgtatcaaggaacgcatgatgaaagagggctcgatgatggttacgtaccaggcacagaagggccacccgaattttttccgtattgtgttccaaaatagcggactcgataaagctgatatggtccaccttgtcgaagagatcgaacggcttggttcagatttgtaa

SEQ ID NO: 71 - DNA, 1623 bp, synthetic construct
  misc_feature 1..1623: note = synthetic_gene coding tcPanD F139G (var.)
  source 1..1623: mol_type = other DNA
atgccggcaaccggagaggaccaagacttggttcaggacttgatcgaggaacctgccactttcagcgacgctgtgttgtcctccgacgaggaactgtttcaccagaaatgcccgaagccggcaccaatttactcgccagtgtcaaaacccgtttcattcgagagcctgcccaatcgccgccttcatgaagaatttctccgctcatcggttgatgtactcctgcaggaggccgttttcgagggaactaatcggaagaatcgggtgcttcagtggcgtgagccagaggaattgcggcgtctcatggattttggcgttcggtctgctccttcaacccacgaagaactgctggaagttcttaaaaaagtagtcacgtacagcgtcaagaccggccacccctactttgtaaatcaactcggtagcgctgtcgacccctatggcctggtcgcgcaatgggctaccgatgccttgaatccctcagtgtacacgtacgaagttagcccggtcttcgtccttatggaggaagtcgtcctgcgtgaaatgcgtgcgattgtcggctttgagggaggcaagggagacggaattttctgtccaggtggctctatcgccaacggttacgcaatttcgtgtgcacggtatcgtttcatgccggatattaagaaaaaaggactgcactcacttccacggctggtactcttcacctcggaagacgctcactactcgatcaaaaaactggcatccttccagggcatcggcaccgataacgtttaccttatccgtactgatgcacggggccggatggatgtttctcacctggtggaggaaattgagcgctcgttgcgtgagggtgccgccccgttcatggtatccgccaccgcaggtacgacggtgatcggagcttttgaccctatcgaaaagatcgccgatgtctgccagaaatacaaattgtggctccacgttgacgctgcctggggtggaggagccttggtctcggctaagcatcgccatctgctcaaaggcatcgagcgggctgattctgttacgtggaatcctcataaactgcttaccgcaccccaacagtgcagcactttgcttcttcgccatgaaggcgtactggcggaagcacatagcaccaatgctgcttacctgttccagaaggacaagttttacgacaccaaatacgacaccggcgataaacacatccaatgtggtcggcgtgccgacgtgttgaaattctggttcatgtggaaggctaaaggcacctccggcttggaaaaacacgttgataaggtatttgaaaacgctcggttctttaccgactgtattaaaaaccgtgagggattcgagatggtaattgctgagccagagtatacgaacatctgtttctggtacgtaccaaaatccctgcggggccggaaggatgaagctgattataaagacaaattgcataaagtcgctccacgtatcaaggaacgcatgatgaaagagggctcgatgatggttacgtaccaggcacagaagggccacccgaattttttccgtattgtgttccaaaatagcggactcgataaagctgatatggtccaccttgtcgaagagatcgaacggcttggttcagatttgtaa

SEQ ID NO: 72 - DNA, 1623 bp, synthetic construct
  misc_feature 1..1623: note = synthetic_gene coding tcPanD F139H (var.)
  source 1..1623: mol_type = other DNA
atgccggcaaccggagaggaccaagacttggttcaggacttgatcgaggaacctgccactttcagcgacgctgtgttgtcctccgacgaggaactgtttcaccagaaatgcccgaagccggcaccaatttactcgccagtgtcaaaacccgtttcattcgagagcctgcccaatcgccgccttcatgaagaatttctccgctcatcggttgatgtactcctgcaggaggccgttttcgagggaactaatcggaagaatcgggtgcttcagtggcgtgagccagaggaattgcggcgtctcatggattttggcgttcggtctgctccttcaacccacgaagaactgctggaagttcttaaaaaagtagtcacgtacagcgtcaagaccggccacccctactttgtaaatcaactccatagcgctgtcgacccctatggcctggtcgcgcaatgggctaccgatgccttgaatccctcagtgtacacgtacgaagttagcccggtcttcgtccttatggaggaagtcgtcctgcgtgaaatgcgtgcgattgtcggctttgagggaggcaagggagacggaattttctgtccaggtggctctatcgccaacggttacgcaatttcgtgtgcacggtatcgtttcatgccggatattaagaaaaaaggactgcactcacttccacggctggtactcttcacctcggaagacgctcactactcgatcaaaaaactggcatccttccagggcatcggcaccgataacgtttaccttatccgtactgatgcacggggccggatggatgtttctcacctggtggaggaaattgagcgctcgttgcgtgagggtgccgccccgttcatggtatccgccaccgcaggtacgacggtgatcggagcttttgaccctatcgaaaagatcgccgatgtctgccagaaatacaaattgtggctccacgttgacgctgcctggggtggaggagccttggtctcggctaagcatcgccatctgctcaaaggcatcgagcgggctgattctgttacgtggaatcctcataaactgcttaccgcaccccaacagtgcagcactttgcttcttcgccatgaaggcgtactggcggaagcacatagcaccaatgctgcttacctgttccagaaggacaagttttacgacaccaaatacgacaccggcgataaacacatccaatgtggtcggcgtgccgacgtgttgaaattctggttcatgtggaaggctaaaggcacctccggcttggaaaaacacgttgataaggtatttgaaaacgctcggttctttaccgactgtattaaaaaccgtgagggattcgagatggtaattgctgagccagagtatacgaacatctgtttctggtacgtaccaaaatccctgcggggccggaaggatgaagctgattataaagacaaattgcataaagtcgctccacgtatcaaggaacgcatgatgaaagagggctcgatgatggttacgtaccaggcacagaagggccacccgaattttttccgtattgtgttccaaaatagcggactcgataaagctgatatggtccaccttgtcgaagagatcgaacggcttggttcagatttgtaa

SEQ ID NO: 73 - DNA, 34 bp, synthetic construct
  misc_feature 1..34: note = synthetic_primer
  source 1..34: mol_type = other DNA
attcgagctcggtaccctggcctcacggatcgtg

SEQ ID NO: 74 - DNA, 34 bp, synthetic construct
  misc_feature 1..34: note = synthetic_primer
  source 1..34: mol_type = other DNA
ggcgagctaaaacgcccggggtcctgtggtgtcc

SEQ ID NO: 75 - DNA, 30 bp, synthetic construct
  misc_feature 1..30: note = synthetic_primer
  source 1..30: mol_type = other DNA
ccacaggaccccgggcgttttagctcgcca

SEQ ID NO: 76 - DNA, 31 bp, synthetic construct
  misc_feature 1..31: note = synthetic_primer
  source 1..31: mol_type = other DNA
cgactctagaggatccccgacgccctcgatc

SEQ ID NO: 77 - DNA, 14 bp, synthetic construct
  misc_feature 1..14: note = synthetic_primer
  source 1..14: mol_type = other DNA
atgccggcaaccgg

SEQ ID NO: 78 - DNA, 31 bp, synthetic construct
  misc_feature 1..31: note = synthetic_primer
  source 1..31: mol_type = other DNA
ggcgagctaaaacgcccttacaaatctgaac

SEQ ID NO: 79 - DNA, 33 bp, synthetic construct
  misc_feature 1..33: note = synthetic_primer
  source 1..33: mol_type = other DNA
aggacaccacaggaccccttcagggtagttgac

SEQ ID NO: 80 - DNA, 33 bp, synthetic construct
  misc_feature 1..33: note = synthetic_primer
  source 1..33: mol_type = other DNA
ctccggttgccggcatctttgtgcacctttcga

SEQ ID NO: 81 - DNA, 16 bp, synthetic construct
  misc_feature 1..16: note = synthetic_primer
  source 1..16: mol_type = other DNA
tctagatcagcgattg

SEQ ID NO: 82 - DNA, 16 bp, synthetic construct
  misc_feature 1..16: note = synthetic_primer
  source 1..16: mol_type = other DNA
gagatcgcgcactaac

SEQ ID NO: 83 - DNA, 26 bp, synthetic construct
  misc_feature 1..26: note = synthetic_primer
  source 1..26: mol_type = other DNA
ggtcgacagcgctgtagagttgattt

SEQ ID NO: 84 - DNA, 28 bp, synthetic construct
  misc_feature 1..28: note = synthetic_primer
  source 1..28: mol_type = other DNA
tttgtaaatcaactctacagcgctgtcg